European Patent Application EP 4 733 768 A2, published April 29, 2026. Title: Thermodynamic Prediction. Applicant: University of Edinurgh. The sequence listing filed with the application follows.

SEQUENCE LISTING (49 sequences)

SEQ ID NO: 1 - protein, 35 aa, Coronavirus
RITFGGPSDSTGSNQNGERSGARSKQRRPQGLPNN

SEQ ID NO: 2 - protein, 12 aa, Coronavirus
QLPQGTTLPKGF

SEQ ID NO: 3 - protein, 30 aa, Coronavirus
EGSRGGSQASSRSSSRSRNSSRNSTPGSSR

SEQ ID NO: 4 - protein, 36 aa, Coronavirus
NSSRNSTPGSSRGTSPARMAGNGGDAALALLLLDRL

SEQ ID NO: 5 - protein, 34 aa, Coronavirus
ALALLLLDRLNQLESKMSGKGQQQQGQTVTKKSA

SEQ ID NO: 6 - protein, 15 aa, Coronavirus
AALALLLLDRLNQLE

SEQ ID NO: 7 - protein, 15 aa, Coronavirus
KTFPPTEPKKDKKKK

SEQ ID NO: 8 - protein, 40 aa, Coronavirus
QALPQRQKKQQTVTLLPAADLDDFSKQLQQSMSSADSTQA

SEQ ID NO: 9 - protein, 19 aa, Coronavirus
MADSNGTITVEELKKLLEQ

SEQ ID NO: 10 - protein, 73 aa, Coronavirus
HRSYLTPGDSSSGWTAGAAAYYVGYLQPRTFLLKYNENGTITDAVDCALDPLSETKCTLKSFTVEKGIYQTSN

SEQ ID NO: 11 - protein, 36 aa, Coronavirus
LTESNKKFLPFQQFGRDIADTTDAVRDPQTLEILDI

SEQ ID NO: 12 - protein, 23 aa, Coronavirus
SNKKFLPFQQFGRDIADTTDAVR

SEQ ID NO: 13 - protein, 16 aa, Coronavirus
QTQTNSPRRARSVASQ

SEQ ID NO: 14 - protein, 20 aa, Coronavirus
LPDPSKPSKRSFIEDLLFNK

SEQ ID NO: 15 - protein, 30 aa, Coronavirus
DPLQPELDSFKEELDKYFKNHTSPDVDLGD

SEQ ID NO: 16 - protein, 72 aa, Coronavirus
FTTAPAICHDGKAHFPREGVFVSNGTHWFVTQRNFYEPQIITTDNTFVSGNCDVVIGIVNNTVYDPLQPELD

SEQ ID NO: 17 - protein, 20 aa, Coronavirus
PRMCSLMQGSTLPRRSGAAG

SEQ ID NO: 18 - protein, 20 aa, synthetic construct
GGGGSPKPSTPPGSSGGGGS

SEQ ID NO: 19 - protein, 5 aa, synthetic construct
GGGGS

SEQ ID NO: 20 - protein, 158 aa, synthetic construct
SQALPQRQKKQQTVTLLPAADLDDFSKQLQQSMSSADSTQASGSSETPGTAEDGGLQLPQGTTLPKGFYALASGDGSGASPGLGLTESNKKFLPFQQFGRDIADTTDAVRDPQTLEILDISGSRWPAGHLPGGLPDPSKPSKRSFIEDLLFNKVTLAG

SEQ ID NO: 21 - protein, 180 aa, synthetic construct
QLPQGTTLPKGFGSSGSRWGPAGHLPGGQALPQRQKKQQTVTLLPAADLDDFSKQLQQSMSSADSTQAALASGDAAVASPGLGRITFGGPSDSTGSNQNGERSGARSKQRRPQGLPNNGLGGAAASTGKTFPPTEPKKDKKKKAGGRSAGGAGNGGDAALALLLLDRLNQLESKMSGLVG

SEQ ID NO: 22 - protein, 238 aa, synthetic construct
MADSNGTITVEELKKLLEQGGGGSPKPSTPPGSSGGGGSRITFGGPSDSTGSNQNGERSGARSKQRRPQGLPNNGGGGSPKPSTPPGSSGGGGSQLPQGTTLPKGFGGGGSPKPSTPPGSSGGGGSAALALLLLDRLNQLEGGGGSPKPSTPPGSSGGGGSKTFPPTEPKKDKKKKGGGGSPKPSTPPGSSGGGGSQALPQRQKKQQTVTLLPAADLDDFSKQLQQSMSSADSTQAGS

SEQ ID NO: 23 - protein, 449 aa, synthetic construct
MADSNGTITVEELKKLLEQGGGGSPKPSTPPGSSGGGGSRITFGGPSDSTGSNQNGERSGARSKQRRPQGLPNNGGGGSPKPSTPPGSSGGGGSQLPQGTTLPKGFGGGGSPKPSTPPGSSGGGGSAALALLLLDRLNQLEGGGGSPKPSTPPGSSGGGGSQALPQRQKKQQTVTLLPAADLDDFSKQLQQSMSSADSTQAGGGGSPKPSTPPGSSGGGGSLTESNKKFLPFQQFGRDIADTTDAVRDPQTLEILDIGGGGSPKPSTPPGSSGGGGSLPDPSKPSKRSFIEDLLFNKGGGGSPKPSTPPGSSGGGGSFTTAPAICHDGKAHFPREGVFVSNGTHWFVTQRNFYEPQIITTDNTFVSGNCDVVIGIVNNTVYDPLQPELDSFKEELDKYFKNHTSPDVDLGDGGGGSPKPSTPPGSSGGGGSQTQTNSPRRAPSVASQGS

SEQ ID NO: 24 - protein, 280 aa, synthetic construct
MADSNGTITVEELKKLLEQGGGGSPKPSTPPGSSGGGGSRITFGGPSDSTGSNQNGERSGARSKQRRPQGLPNNGGGGSPKPSTPPGSSGGGGSQALPQRQKKQQTVTLLPAADLDDFSKQLQQSMSSADSTQAGGGGSPKPSTPPGSSGGGGSLTESNKKFLPFQQFGRDIADTTDAVRDPQTLEILDIGGGGSPKPSTPPGSSGGGGSLPDPSKPSKRSFIEDLLFNKGGGGSPKPSTPPGSSGGGGSDPLQPELDSFKEELDKYFKNHTSPDVDLGD

SEQ ID NO: 25 - protein, 228 aa, synthetic construct
LTESNKKFLPFQQFGRDIADTTDAVRDPQTLEILDIGGGGSPKPSTPPGSSGGGGSLPDPSKPSKRSFIEDLLFNKGGGGSPKPSTPPGSSGGGGSQTQTNSPRRAPSVASQGGGGSPKPSTPPGSSGGGGSFTTAPAICHDGKAHFPREGVFVSNGTHWFVTQRNFYEPQIITTDNTFVSGNCDVVIGIVNNTVYDPLQPELDSFKEELDKYFKNHTSPDVDLGDGS

SEQ ID NO: 26 - protein, 163 aa, synthetic construct
MADSNGTITVEELKKLLEQGGGGSRITFGGPSDSTGSNQNGERSGARSKQRRPQGLPNNGGGGSQLPQGTTLPKGFGGGGSAALALLLLDRLNQLEGGGGSKTFPPTEPKKDKKKKGGGGSQALPQRQKKQQTVTLLPAADLDDFSKQLQQSMSSADSTQAGS

SEQ ID NO: 27 - protein, 329 aa, synthetic construct
MADSNGTITVEELKKLLEQGGGGSRITFGGPSDSTGSNQNGERSGARSKQRRPQGLPNNGGGGSQLPQGTTLPKGFGGGGSAALALLLLDRLNQLEGGGGSQALPQRQKKQQTVTLLPAADLDDFSKQLQQSMSSADSTQAGGGGSLTESNKKFLPFQQFGRDIADTTDAVRDPQTLEILDIGGGGSLPDPSKPSKRSFIEDLLFNKGGGGSQTQTNSPRRAPSVASQGGGGSFTTAPAICHDGKAHFPREGVFVSNGTHWFVTQRNFYEPQIITTDNTFVSGNCDVVIGIVNNTVYDPLQPELDSFKEELDKYFKNHTSPDVDLGDGS

SEQ ID NO: 28 - protein, 205 aa, synthetic construct
MADSNGTITVEELKKLLEQGGGGSRITFGGPSDSTGSNQNGERSGARSKQRRPQGLPNNGGGGSQALPQRQKKQQTVTLLPAADLDDFSKQLQQSMSSADSTQAGGGGSLTESNKKFLPFQQFGRDIADTTDAVRDPQTLEILDIGGGGSLPDPSKPSKRSFIEDLLFNKGGGGSDPLQPELDSFKEELDKYFKNHTSPDVDLGD

SEQ ID NO: 29 - protein, 182 aa, synthetic construct
LTESNKKFLPFQQFGRDIADTTDAVRDPQTLEILDIGGGGSLPDPSKPSKRSFIEDLLFNKGGGGSQTQTNSPRRAPSVASQGGGGSFTTAPAICHDGKAHFPREGVFVSNGTHWFVTQRNFYEPQIITTDNTFVSGNCDVVIGIVNNTVDPLQPELDSFKEELDKYFKNHTSPDVDLGDGS

SEQ ID NO: 30 - protein, 61 aa, Epstein Barr Virus
LTELTTPTSSPPSSPSPPAPSAARGSTPAAVLRRRRRDAGNATTPVPPTAPGKSLGTLNNP

SEQ ID NO: 31 - protein, 22 aa, Epstein Barr Virus
PKFQELNQNNLPNDVFREAQRS

SEQ ID NO: 32 - protein, 53 aa, Epstein Barr Virus
RLEPWQPLPGPQVTAVLLHEESMQGVQVHGSMLDLLEKDDEVMEQRVMATLLP

SEQ ID NO: 33 - protein, 36 aa, Epstein Barr Virus
PWRPEPNTSSPSMPELSPVLGLHQGQGAGDSPTPGP

SEQ ID NO: 34 - protein, 19 aa, Epstein Barr Virus
PEWPVQGESGQNVTDHEPR

SEQ ID NO: 35 - protein, 38 aa, Epstein Barr Virus
GASGSEDPPDYGDQGNVQQVGSGPISPEIGPFELSAAS

SEQ ID NO: 36 - protein, 54 aa, Epstein Barr Virus
SEGPGPTRPGPPGIGPEGPLGQLLRRHRSPSPTRGGQEPRRVRRRVLVQQEEEV

SEQ ID NO: 37 - protein, 19 aa, Epstein Barr Virus
VIIIWKLLRTKFGRKPRLI

SEQ ID NO: 38 - protein, 19 aa, Epstein Barr Virus
PRKVRLPSVKAVDMSMEDM

SEQ ID NO: 39 - protein, 28 aa, Epstein Barr Virus
EEGRACGETNEGLEYDEDSENDELLFLP

SEQ ID NO: 40 - protein, 41 aa, Epstein Barr Virus
GAKGQPSPGEGTRPRESNDPNATRRARSRSRGREAKKVQIS

SEQ ID NO: 41 - protein, 36 aa, Epstein Barr Virus
GSSQAAPSFSSVAPVASLSGDLEEEEEGSRESPSLP

SEQ ID NO: 42 - protein, 39 aa, Epstein Barr Virus
RVIGDEDEDGSEDGEFSDLDLSDSDHEGDEGGGAVGGGR

SEQ ID NO: 43 - protein, 63 aa, Epstein Barr Virus
PSSQSSSSGSPPRRPPPGRRPFFHPVGEADYFEYHQEGGPDGEPDVPPGAIEQGPADDPGEGP

SEQ ID NO: 44 - protein, 24 aa, Epstein Barr Virus
RTNYKIVDYDNRGTNPQGERRAFL

SEQ ID NO: 45 - protein, 10 aa, Epstein Barr Virus
LWNLHGQALF

SEQ ID NO: 46 - protein, 19 aa, Coronavirus
MANSNGTITVEELKKLLEE

SEQ ID NO: 47 - protein, 19 aa, Coronavirus
MADSNGTITVEELKKLLEE

SEQ ID NO: 48 - protein, 19 aa, Coronavirus
MAGSNGTITVEELKKLLEE

SEQ ID NO: 49 - protein, 19 aa, Coronavirus
MAYSNGTITVEELKKLLEE